European Patent Application EP 4 537 850 A1, published April 16, 2025. Title: 보툴리눔 독소 안정화 조성물, 이를 포함하는 보툴리눔 독소 제제 및 이에 사용하기 위한 폴리펩티드. Applicant: (주)메디톡스. The sequence listing filed with the application follows.

SEQUENCE LISTING (24 sequences)

SEQ ID NO: 1 - protein, 10 aa, Artificial Sequence
RRLQQTQAQV

SEQ ID NO: 2 - protein, 11 aa, Artificial Sequence
RRLQQTQAQVD

SEQ ID NO: 3 - protein, 12 aa, Artificial Sequence
RRLQQTQAQVDE

SEQ ID NO: 4 - protein, 13 aa, Artificial Sequence
RRLQQTQAQVDEV

SEQ ID NO: 5 - protein, 14 aa, Artificial Sequence
RRLQQTQAQVDEVV

SEQ ID NO: 6 - protein, 15 aa, Artificial Sequence
RRLQQTQAQVDEVVD

SEQ ID NO: 7 - protein, 16 aa, Artificial Sequence
RRLQQTQAQVDEVVDI

SEQ ID NO: 8 - protein, 17 aa, Artificial Sequence
RRLQQTQAQVDEVVDIM

SEQ ID NO: 9 - protein, 17 aa, Artificial Sequence
RRLQQTQAQVDEVVDIA

SEQ ID NO: 10 - protein, 17 aa, Artificial Sequence
RRLQQAQAQVDEVVDIM

SEQ ID NO: 11 - protein, 15 aa, Artificial Sequence
RRWRRWNRFNRRRCR

SEQ ID NO: 12 - protein, 9 aa, Artificial Sequence
RRWWRRWRR

SEQ ID NO: 13 - protein, 9 aa, Artificial Sequence
RRRWRRWRR

SEQ ID NO: 14 - protein, 32 aa, Artificial Sequence
RRWRRWNRFNRRRCRRRLQQTQAQVDEVVDIM

SEQ ID NO: 15 - protein, 26 aa, Artificial Sequence
RRWWRRWRRRRLQQTQAQVDEVVDIM

SEQ ID NO: 16 - protein, 25 aa, Artificial Sequence
RRWRRWNRFNRRRCRRRLQQTQAQV

SEQ ID NO: 17 - protein, 26 aa, Artificial Sequence
RRRWRRWRRRRLQQTQAQVDEVVDIM

SEQ ID NO: 18 - protein, 31 aa, Artificial Sequence
RRWRRWNRFNRRRCRGWRFIRIDTSCVCTLT

SEQ ID NO: 19 - protein, 32 aa, Artificial Sequence
RALTMDSKKRIGWRFIRIDTSCVCTLTIKRGR

SEQ ID NO: 20 - protein, 32 aa, Artificial Sequence
RRWRRWNRFNRRRCRRRLQQTQAQVDEVVDIA

SEQ ID NO: 21 - protein, 32 aa, Artificial Sequence
RRWRRWNRFNRRRCRRRLQQAQAQVDEVVDIM

SEQ ID NO: 22 - protein, 35 aa, Artificial Sequence
RKKRRQRRRGKKKKKKKKKKKKKKKGRKKRRQRRR

SEQ ID NO: 23 - protein, 425 aa, Artificial Sequence
MPFVNKQFNYKDPVNGVDIAYIKIPNAGQMQPVKAFKIHNKIWVIPERDTFTNPEEGDLNPPPEAKQVPVSYYDSTYLSTDNEKDNYLKGVTKLFERIYSTDLGRMLLTSIVRGIPFWGGSTIDTELKVIDTNCINVIQPDGSYRSEELNLVIIGPSADIIQFECKSFGHEVLNLTRNGYGSTQYIRFSPDFTFGFEESLEVDTNPLLGAGKFATDPAVTLAHELIHAGHRLYGIAINPNRVFKVNTNAYYEMAGLEVSLEELITFGGNDAKFIDSLQKKEFSLYYYNKFKDIASTLNKAKSIVGTTASLQYMKNVFKEKYLLSEDATGKFLVDRLKFDELYKLLTEIYTEDNFVKFFKVLNRKTYLNFDKAVFKINIVPDVNYTIHDGFNLRNTNLAANFNGQNIEINNKNFDKLKNFTGLFEF

SEQ ID NO: 24 - protein, 1296 aa, Artificial Sequence
MPFVNKQFNYKDPVNGVDIAYIKIPNAGQMQPVKAFKIHNKIWVIPERDTFTNPEEGDLNPPPEAKQVPVSYYDSTYLSTDNEKDNYLKGVTKLFERIYSTDLGRMLLTSIVRGIPFWGGSTIDTELKVIDTNCINVIQPDGSYRSEELNLVIIGPSADIIQFECKSFGHEVLNLTRNGYGSTQYIRFSPDFTFGFEESLEVDTNPLLGAGKFATDPAVTLAHELIHAGHRLYGIAINPNRVFKVNTNAYYEMAGLEVSLEELITFGGNDAKFIDSLQKKEFSLYYYNKFKDIASTLNKAKSIVGTTASLQYMKNVFKEKYLLSEDATGKFLVDRLKFDELYKLLTEIYTEDNFVKFFKVLNRKTYLNFDKAVFKINIVPDVNYTIHDGFNLRNTNLAANFNGQNIEINNKNFDKLKNFTGLFEFYKLLCVRGIITSKTKSLDKGYNKALNDLCIKVNNWDLFFSPSEDNFTNDLNKGEEITSDTNIEAAEENISLDLIQQYYLTFNFDNEPENISIENLSSDIIGQLELMPNIERFPNGKKYELDKYTMFHYLRAQEFEHGKSRIALTNSVNEALLNPSRVYTFFSSDYVKKVNKATEAAMFLGWVEQLVYDFTDETSEVSTTDKIADITIIIPYIGPALNIGNMLYKDDFVGALIFSGAVILLEFIPEIAIPVLGTFALVSYIANKVLTVQTIDNALSKRNEKWDEVYKYIVTNWLAKVNTQIDLIRKKMKEALENQAEATKAIINYQYNQYTEEEKNNINFNIDDLSSKLNESINKAMININKFLNQCSVSYLMNSMIPYGVKRLEDFDASLKDALLKYIYDNRGTLIGQVDRLKDKVNNTLSTDIPFQLSKYVDNQRLLSTFTEYIKNIINTSILNLRYESNHLIDLSRYASKINIGSKVNFDPIDKNQIQLFNLESSKIEVILKNAIVYNSMYENFSTSFWIRIPKYFNSISLNNEYTIINCMENNSGWKVSLNYGEIIWTLQDTQEIKQRVVFKYSQMINISDYINRWIFVTITNNRLNNSKIYINGRLIDQKPISNLGNIHASNNIMFKLDGCRDTHRYIWIKYFNLFDKELNEKEIKDLYDNQSNSGILKDFWGDYLQYDKPYYMLNLYDPNKYVDVNNVGIRGYMYLKGPRGSVMTTNIYLNSSLYRGTKFIIKKYASGNKDNIVRNNDRVYINVVVKNKEYRLATNASQAGVEKILSALEIPDVGNLSQVVVMKSKNDQGITNKCKMNLQDNNGNDIGFIGFHQFNNIAKLVASNWYNRQIERSSRTLGCSWEFIPVDDGWGERPL